European Patent Specification EP 3 672 987 B1, published April 16, 2025. Title: Anti-apelin Antibodies and Uses Thereof. Applicant: Phanes Therapeutics, Inc. The sequence listing filed with the application follows.

SEQUENCE LISTING (221 sequences)

SEQ ID NO: 1 - protein, 113 aa, Artificial Sequence
  C8 Heavy Chain Variable Region
QSVEESGGRLVTPGTPLTLTCTVSGIDLYSNRMSWVRQAPGKGLEWIGSIGSSPWYASWAQGRFTISKTSSTTVNLKITSPTTEDTATYFCAKGGYRPGASVWGPGTLVTVSS

SEQ ID NO: 2 - protein, 109 aa, Artificial Sequence
  C8 Light Chain Variable Region
QVLTQTESPVSAPVGGTVTIACQSSQSVYDNNDLAWYQQKAGQTPKRLIYLASSLDSGVPSRFKGSGSGTEFTLTISDLECDDAATYYCAGGYSGDIYTFGGGTEVVVE

SEQ ID NO: 3 - protein, 112 aa, Artificial Sequence
  C24 Heavy Chain Variable Region
QSLEESGGRLVTPGTPLTLTCTVSGIDLYTNRVSWVRQAPGKGLDWIGSIGSSPWYASWAQGRFTISKTSTTVNLKITSSTTEDTATYFCAKGGYRPGGSIWGPGTLVTVSS

SEQ ID NO: 4 - protein, 109 aa, Artificial Sequence
  C24 Light Chain Variable Region
QVLTQSASPVSAAVGDSVTIACQSSQSVYDNNDLGWYQQKPGQTPKRLIYLASSLDSGVPSRFSGSGSGTQFTLTISDLECDDAATYYCAGGYSGDIYTFGGGTEVVVK

SEQ ID NO: 5 - protein, 112 aa, Artificial Sequence
  C25 Heavy Chain Variable Region
QSLEESGGGLVTPGTPLTLTCTVSGIDLYTNRMSWVRQAPGKGLEWIGSIGSSPWFASWALGRFTISKTSTTVNLKITSPTTEDTATYFCAKGGYRPGASVWGPGTLVTVSS

SEQ ID NO: 6 - protein, 109 aa, Artificial Sequence
  C25 Light Chain Variable Region
QVLTQTESPVSAPVGGTVTIACQSSQSVYDNNDLAWYQQKAGQTPKRLIFLASSLDSGVPSRFKGSGSGTEFTLTISDLECDDAATYYCAGGYNGDIYTFGGGTEVVVK

SEQ ID NO: 7 - protein, 115 aa, Artificial Sequence
  C7 Heavy Chain Variable Region
QSLEESGGRLAKPDETLTLTCTVSGIDLNSHAMDWVRQAPGKGLEWIGVIAPDTRTYYATWARGRFTISKTSSTSVELKMTSLTTEDTATYFCAAYPIEPGANIWGPGTLVTVSS

SEQ ID NO: 8 - protein, 110 aa, Artificial Sequence
  C7 Light Chain Variable Region
DPVLTQTPSPVSAPVGGTVTIGCQASESVDYNNQLSWYQQKPGQAPKRLMYYVSTLDSGVPSRFKGSGSGTQFTLTISDLECDDAATYYCQGGYPYNIYPFGGGTEVVVK

SEQ ID NO: 9 - protein, 115 aa, Artificial Sequence
  C6 Heavy Chain Variable Region
QSLEESGGRLVKPDETLTLTCTVSGIDLSNYAMDWVRQAPGKGLEWIGVIAPNRRTYYPTWARGRFTISKTSSTTVDLKMTSLTTEDTATYFCATYPIEPGANIWGPGTLVTVSS

SEQ ID NO: 10 - protein, 110 aa, Artificial Sequence
  C6 Light Chain Variable Region
DPVLTQTPSPVSAPVGGTVTIGCQSSESVDYNNQLSWYQQKPGQPPKRLMYYVSTLDSGVPSRFKGSGSGTQFTLTISDLECDDAATYYCQGGYISNIYPFGGGTEVVVK

SEQ ID NO: 11 - protein, 114 aa, Artificial Sequence
  C1 Heavy Chain Variable Region
QSLEESGGRLVTPGGSLTLTCTVSGFSLSSYAMDWVRQAPGKGLEWIGVIAPNGATYYPTWARGRFTISKTSTTVDLKMTSLTAADTATYFCATYPIDAGANIWGPGTLVTVSS

SEQ ID NO: 12 - protein, 110 aa, Artificial Sequence
  C1 Light Chain Variable Region
DPVLTQTPSSVSAAVGGTVTIGCQSSESVDNNNQLSWYQQKSGQPPKRLMYYVSTLDSGVPSRFKGSGSGTHFTLTISGVQCYDAATYYCQGGYISNLYPFGGGTEVVVK

SEQ ID NO: 13 - protein, 114 aa, Artificial Sequence
  C16 Heavy Chain Variable Region
QSLEESGGRLVTPGGSLTLTCTVSGIDLNSYAMDWVRQAPGKGLEWIGVIAPNHYTYYPTWARGRFTISKTSTTVDLKMTRLTTEDTATYFCATYPIESGSNIWGPGTLVIVSS

SEQ ID NO: 14 - protein, 110 aa, Artificial Sequence
  C16 Light Chain Variable Region
DPVLTQTPSSVSAAVGGTVTIGCQSSESVGMNNQLSWYQQKPGQPPKRLMYYVSTLDSGVPSRFKGSGSGTQFSLTISDLECDDAGTYYCQGGYISNLYPFGGGTEVVVK

SEQ ID NO: 15 - protein, 114 aa, Artificial Sequence
  C20 Heavy Chain Variable Region
QSLEESGGRLVTPGGSLTLTCTVSGIDLNNYAIDWVRQAPGKGLEWIGVIAPNHYTCYPTWARGRFTISKTSTTVDLKMTSLTTEDTATYFCAAYPIETGSNIWGPGTLVIVSS

SEQ ID NO: 16 - protein, 110 aa, Artificial Sequence
  C20 Light Chain Variable Region
DPMLTQTPSSVSAAVGGTVTISCQSSESVDMNNQLSWYQQKPGQPPKRLMYYVSTLDSGVPSRFKGSGSGIHFSLTISDLECADAGTYYCQGGYISNLYPFGGGTEVVVK

SEQ ID NO: 17 - protein, 114 aa, Artificial Sequence
  C22 Heavy Chain Variable Region
QSLEESGGRLVTPGGSLTLTCTVSGIDLNNYAMDWVRQAPGKGLEWIGVIAPNHYTYYPTWARGRFTISKTSTTVDLKMTSLTTEDTATYFCATYPIETGSNIWGPGTLVIVSS

SEQ ID NO: 18 - protein, 110 aa, Artificial Sequence
  C22 Light Chain Variable Region
DPVLTQTPSSVSAAVGGTVTISCQSSESVDMNNQLSWYHQKSGQPPKRLMYYVSTLDSGVPSRFKGSGSGTQFTLTISGVQCDDAGTYYCQGGYISNLYPFGGGTEVVVK

SEQ ID NO: 19 - protein, 114 aa, Artificial Sequence
  C10 Heavy Chain Variable Region
QSLEESGGRLVTPGGSLTLTCTVSGIDLNSYAIDWVRQAPGKGLEWIGVIAPSGTTYYPTWAKGRFTISKTSTTVDLKVTGLTTEDTATYFCAAYPIDPGSNIWGPGTLVTVSS

SEQ ID NO: 20 - protein, 110 aa, Artificial Sequence
  C10 Light Chain Variable Region
DPVLTQTPSSVSAAVGGTATIGCQSSESVDYGNQLSWYQQKPGQPPKRLAYYVSILDAGVPSRFKGSGSGTQFTLTISDLECDDAATYYCQGGYISNLYPFGGGTEVVVQ

SEQ ID NO: 21 - protein, 115 aa, Artificial Sequence
  C12 Heavy Chain Variable Region
QSLEESGGRLVTPGGSLTLTCTVSGIDLSSYAIDWVRQAPGKGLEWIGVIAPSSTTYYPTWAKGRFTISKTSSTTVDLKVIGLTTEDTATYFCAAYPIDPGSNVWGPGTLVTVSS

SEQ ID NO: 22 - protein, 110 aa, Artificial Sequence
  C12 Light Chain Variable Region
DPVLTQTPSSVSAAVGGTVTIGCQSSESVDYGNQLSWYQQKPGQPPKRLTYYVSILDAGVPSRFKGSGSGTQFTLTISDLECDDAATYYCQGGYISNLYPFGGGTEVVVQ

SEQ ID NO: 23 - protein, 115 aa, Artificial Sequence
  C13 Heavy Chain Variable Region
QSLEESGGRLAKPGETLTLTCTVSGIDLNSHAVDWVRQAPGKGLEWIGVIGPGGNTYYASWAKGRFTISKTSSTTVDLKMTSLTAEDTATFFCATYPIYSGDNIWGPGTLVTVSS

SEQ ID NO: 24 - protein, 110 aa, Artificial Sequence
  C13 Light Chain Variable Region
DPVLTQTPPSVSAAVGGTVTINCQSSESVDNNNQLSWYQQKVGQPPKRLMYYASTLDSGVPSRFKGGGSGTHFTLTITDLECDDAATYYCQGGTATNIYPFGGGTEVVVK

SEQ ID NO: 25 - protein, 114 aa, Artificial Sequence
  C14 Heavy Chain Variable Region
QSPEESGGRLVTPGGSLTLTCKISGVDLSNYAMDWVRQAPGKGLEWIGVIAPNDATYYPTWARGRLTISKTSTTVDLKMTRLTTEDTATYFCAAYPIDVGANVWGPGTLVTVSS

SEQ ID NO: 26 - protein, 110 aa, Artificial Sequence
  C14 Light Chain Variable Region
DPMLTQTASPVSAAVGGTVTINCQSSESVDYNNQLSWYQQKPGQPPKRLMYYVSTLDSGVPSRFKGSGSGTQFSLTISDLECDDAGTYYCQGGYISNLYPFGGGTEVVVK

SEQ ID NO: 27 - protein, 114 aa, Artificial Sequence
  C11 Heavy Chain Variable Region
QSLEESGGRLVSPGGSLTLTCTVSGIDLSSHAMDWVRQAPGKGLEWIGVIAPNDATYYPTWARGRFTISKTSTTVGLKMTRLTTEDTATYFCAAYPIDAGANVWGPGTLVTVSS

SEQ ID NO: 28 - protein, 110 aa, Artificial Sequence
  C11 Light Chain Variable Region
DPMLTQTASPVSAHVGGTVTINCQSSESVDYNNQLSWYQQKPGQPPKRLMYYVSTLDSGVPSRFKGSGSGTQFSLTISDLECDDAGTYYCQGGYISNLYPFGGGTEVVVK

SEQ ID NO: 29 - protein, 125 aa, Artificial Sequence
  C4 Heavy Chain Variable Region
QEQLEQSGGGAEGGLVKPGGSLELCCKASGFTLSSSYWICWVRQAPGKGLEWIGCIHYGSSGTAYYASWVNGRFTLSRDIDQSTGCLQLNSLTAADTAMYYCARFLSDMYYYNLWGPGTLVTVSS

SEQ ID NO: 30 - protein, 112 aa, Artificial Sequence
  C4 Light Chain Variable Region
QVLTQTPASVSAAVGGTVTINCQASQSIYNNNQLSWYQQKPGQPPKLLIYYASTLASGVSSRFKGSGSGTQFTLTISGVQCDDAATYYCQGQFNCRSADCHAFGGGTEVVVK

SEQ ID NO: 31 - protein, 110 aa, Artificial Sequence
  C5 Heavy Chain Variable Region
QSVEESGGRLVTPGTPLTLTCTVSGFSLSGAWMNWVRQAPGKGLEWIGVVSSDDNIYYADWAKGRFTISKTSTTVDLKLTSPTTEDTATYFCARNLGTIWGPGTLVTVSS

SEQ ID NO: 32 - protein, 108 aa, Artificial Sequence
  C5 Light Chain Variable Region
QVLTQTESPVSAAVGGTVTINCQSSQSVWSNYLSWFQQKPGQPPKVLIYGTSKLPSGVPSRFSGSGSGTEFTLTINDLECDDAATYYCAGGYSGHIYSFGGGTEVVVK

SEQ ID NO: 33 - protein, 121 aa, Artificial Sequence
  C9 Heavy Chain Variable Region
QEQLEESGGDLVKPEGSLTLTCTASGFSFSSSYWICWVRQAPGKGLEWIACIYQSGDGRTWYASWAEGRFTISKTSPTTVTLQMASLTAADTATYFCARCPHNTYSHFDLWGPSTLVTVSS

SEQ ID NO: 34 - protein, 114 aa, Artificial Sequence
  C9 Light Chain Variable Region
ADIVMTQTPASVEAAVGGTVTIKCQASQSINSWLSWYQQKPGQPPKPLIYGASNLASGVPSRFKGSGSGTQFTLTISDLECADAATYSCLGYYYSSYNSVGFWAFGGGTEVVVK

SEQ ID NO: 35 - protein, 112 aa, Artificial Sequence
  C26 Heavy Chain Variable Region
QEQLEESGGGLVQPEGSLTLTCTASGFTLSNYWMSWVRQAPGKGLVWIGCIDIGSDDTYYASWAKGRFTISRTSSTTVTLQVTSLTAADTATYFCARSGGLWGPGTLVTVSS

SEQ ID NO: 36 - protein, 109 aa, Artificial Sequence
  C26 Light Chain Variable Region
QVLTQTPSSTSAAVGGTVTINCQASQSVYNNNDLAWYQQKPGQPPKRLIYEASKLASGVPSRFSGSGSGTQFTLTISDLECDDAATYYCAGGWSGNFYVFGGGTEVVVK

SEQ ID NO: 37 - protein, 108 aa, Artificial Sequence
  C27 Heavy Chain Variable Region
QSVEESGGRLVTPGGSLTLTCTVSGIDLINAWMNWVRQAPGKGLEWIGTTTDDDTIYYANWAKGRFTISRTSTTVDLKVTSLTSEDTATYFCSKGRIWGPGTLVTVSL

SEQ ID NO: 38 - protein, 109 aa, Artificial Sequence
  C27 Light Chain Variable Region
QVLTQTPASVSAAVGGTVTINCQASQSVYDGNWLCWYQQKPGQPPKRLIYKASTLESGVPSRFKGSGSGTQFTLTISDLECDDAATYYCQGGFTSNIYPFAGGTEVVVK

SEQ ID NO: 39 - protein, 109 aa, Artificial Sequence
  C17 Heavy Chain Variable Region
QSVEESGGRLVKPDETLTLTCAVSGIDLSSNAMNWVRQAPGEGLEWIGSMYTDGTTYYANWAKGRFTISRASSTTVDLKMTSLTAADTATYFCARGDIWGPGTLVTVSS

SEQ ID NO: 40 - protein, 109 aa, Artificial Sequence
  C17 Light Chain Variable Region
QVLTQTASPVSAAVGGTVTISCQSSQSVYNNNWLAWFQQKPGQPPKRLIYGTSELASGVPSRFKGSGSGTQFTLTISGVQCDDAATYYCLGTYSSNIHVFGGGTEVVVK

SEQ ID NO: 41 - protein, 5 aa, Artificial Sequence
  C8 HC CDR1
SNRMS

SEQ ID NO: 42 - protein, 14 aa, Artificial Sequence
  C8 HC CDR2
SIGSSPWYASWAQG

SEQ ID NO: 43 - protein, 9 aa, Artificial Sequence
  C8 HC CDR3
GGYRPGASV

SEQ ID NO: 44 - protein, 5 aa, Artificial Sequence
  C24 HC CDR1
TNRVS

SEQ ID NO: 45 - protein, 14 aa, Artificial Sequence
  C24 HC CDR2
SIGSSPWYASWAQG

SEQ ID NO: 46 - protein, 9 aa, Artificial Sequence
  C24 HC CDR3
GGYRPGGSI

SEQ ID NO: 47 - protein, 5 aa, Artificial Sequence
  C25 HC CDR1
TNRMS

SEQ ID NO: 48 - protein, 14 aa, Artificial Sequence
  C25 HC CDR2
SIGSSPWFASWALG

SEQ ID NO: 49 - protein, 9 aa, Artificial Sequence
  C25 HC CDR3
GGYRPGASV

SEQ ID NO: 50 - protein, 5 aa, Artificial Sequence
  C7 HC CDR1
SHAMD

SEQ ID NO: 51 - protein, 16 aa, Artificial Sequence
  C7 HC CDR2
VIAPDTRTYYATWARG

SEQ ID NO: 52 - protein, 9 aa, Artificial Sequence
  C7 HC CDR3
YPIEPGANI

SEQ ID NO: 53 - protein, 5 aa, Artificial Sequence
  C6 HC CDR1
NYAMD

SEQ ID NO: 54 - protein, 16 aa, Artificial Sequence
  C6 HC CDR2
VIAPNRRTYYPTWARG

SEQ ID NO: 55 - protein, 9 aa, Artificial Sequence
  C6 HC CDR3
YPIEPGANI

SEQ ID NO: 56 - protein, 5 aa, Artificial Sequence
  C1 HC CDR1
SYAMD

SEQ ID NO: 57 - protein, 16 aa, Artificial Sequence
  C1 HC CDR2
VIAPNGATYYPTWARG

SEQ ID NO: 58 - protein, 9 aa, Artificial Sequence
  C1 HC CDR3
YPIDAGANI

SEQ ID NO: 59 - protein, 5 aa, Artificial Sequence
  C16 HC CDR1
SYAMD

SEQ ID NO: 60 - protein, 16 aa, Artificial Sequence
  C16 HC CDR2
VIAPNHYTYYPTWARG

SEQ ID NO: 61 - protein, 9 aa, Artificial Sequence
  C16 HC CDR3
YPIESGSNI

SEQ ID NO: 62 - protein, 5 aa, Artificial Sequence
  C20 HC CDR1
NYAID

SEQ ID NO: 63 - protein, 16 aa, Artificial Sequence
  C20 HC CDR2
VIAPNHYTCYPTWARG

SEQ ID NO: 64 - protein, 9 aa, Artificial Sequence
  C20 HC CDR3
YPIETGSNI

SEQ ID NO: 65 - protein, 5 aa, Artificial Sequence
  C22 HC CDR1
NYAMD

SEQ ID NO: 66 - protein, 16 aa, Artificial Sequence
  C22 HC CDR2
VIAPNHYTYYPTWARG

SEQ ID NO: 67 - protein, 9 aa, Artificial Sequence
  C22 HC CDR3
YPIETGSNI

SEQ ID NO: 68 - protein, 5 aa, Artificial Sequence
  C10 HC CDR1
SYAID

SEQ ID NO: 69 - protein, 16 aa, Artificial Sequence
  C10 HC CDR2
VIAPSGTTYYPTWAKG

SEQ ID NO: 70 - protein, 9 aa, Artificial Sequence
  C10 HC CDR3
YPIDPGSNI

SEQ ID NO: 71 - protein, 5 aa, Artificial Sequence
  C12 HC CDR1
SYAID

SEQ ID NO: 72 - protein, 16 aa, Artificial Sequence
  C12 HC CDR2
VIAPSSTTYYPTWAKG

SEQ ID NO: 73 - protein, 9 aa, Artificial Sequence
  C12 HC CDR3
YPIDPGSNV

SEQ ID NO: 74 - protein, 5 aa, Artificial Sequence
  C13 HC CDR1
SHAVD

SEQ ID NO: 75 - protein, 16 aa, Artificial Sequence
  C13 HC CDR2
VIGPGGNTYYASWAKG

SEQ ID NO: 76 - protein, 9 aa, Artificial Sequence
  C13 HC CDR3
YPIYSGDNI

SEQ ID NO: 77 - protein, 5 aa, Artificial Sequence
  C14 HC CDR1
NYAMD

SEQ ID NO: 78 - protein, 16 aa, Artificial Sequence
  C14 HC CDR2
VIAPNDATYYPTWARG

SEQ ID NO: 79 - protein, 9 aa, Artificial Sequence
  C14 HC CDR3
YPIDVGANV

SEQ ID NO: 80 - protein, 5 aa, Artificial Sequence
  C11 HC CDR1
SHAMD

SEQ ID NO: 81 - protein, 16 aa, Artificial Sequence
  C11 HC CDR2
VIAPNDATYYPTWARG

SEQ ID NO: 82 - protein, 9 aa, Artificial Sequence
  C11 HC CDR3
YPIDAGANV

SEQ ID NO: 83 - protein, 6 aa, Artificial Sequence
  C4 HC CDR1
SSYWIC

SEQ ID NO: 84 - protein, 18 aa, Artificial Sequence
  C4 HC CDR2
CIHYGSSGTAYYASWVNG

SEQ ID NO: 85 - protein, 10 aa, Artificial Sequence
  C4 HC CDR3
FLSDMYYYNL

SEQ ID NO: 86 - protein, 5 aa, Artificial Sequence
  C5 HC CDR1
GAWMN

SEQ ID NO: 87 - protein, 16 aa, Artificial Sequence
  C5 HC CDR2
VVSSDDNIYYADWAKG

SEQ ID NO: 88 - protein, 5 aa, Artificial Sequence
  C5 HC CDR3
NLGTI

SEQ ID NO: 89 - protein, 6 aa, Artificial Sequence
  C9 HC CDR1
SSYWIC

SEQ ID NO: 90 - protein, 18 aa, Artificial Sequence
  C9 HC CDR2
CIYQSGDGRTWYASWAEG

SEQ ID NO: 91 - protein, 11 aa, Artificial Sequence
  C9 HC CDR3
CPHNTYSHFDL

SEQ ID NO: 92 - protein, 5 aa, Artificial Sequence
  C26 HC CDR1
NYWMS

SEQ ID NO: 93 - protein, 17 aa, Artificial Sequence
  C26 HC CDR2
CIDIGSDDTYYASWAKG

SEQ ID NO: 94 - protein, 4 aa, Artificial Sequence
  C26 HC CDR3
SGGL

SEQ ID NO: 95 - protein, 5 aa, Artificial Sequence
  C27 HC CDR1
NAWMN

SEQ ID NO: 96 - protein, 16 aa, Artificial Sequence
  C27 HC CDR2
TTTDDDTIYYANWAKG

SEQ ID NO: 97 - protein, 3 aa, Artificial Sequence
  C27 HC CDR3
GRI

SEQ ID NO: 98 - protein, 5 aa, Artificial Sequence
  C17 HC CDR1
SNAMN

SEQ ID NO: 99 - protein, 16 aa, Artificial Sequence
  C17 HC CDR2
SMYTDGTTYYANWAKG

SEQ ID NO: 100 - protein, 3 aa, Artificial Sequence
  C17 HC CDR3
GDI

SEQ ID NO: 101 - protein, 13 aa, Artificial Sequence
  C8 LC CDR1
QSSQSVYDNNDLA

SEQ ID NO: 102 - protein, 7 aa, Artificial Sequence
  C8 LC CDR2
LASSLDS

SEQ ID NO: 103 - protein, 10 aa, Artificial Sequence
  C8 LC CDR3
AGGYSGDIYT

SEQ ID NO: 104 - protein, 13 aa, Artificial Sequence
  C24 LC CDR1
QSSQSVYDNNDLG

SEQ ID NO: 105 - protein, 7 aa, Artificial Sequence
  C24 LC CDR2
LASSLDS

SEQ ID NO: 106 - protein, 10 aa, Artificial Sequence
  C24 LC CDR3
AGGYSGDIYT

SEQ ID NO: 107 - protein, 13 aa, Artificial Sequence
  C25 LC CDR1
QSSQSVYDNNDLA

SEQ ID NO: 108 - protein, 7 aa, Artificial Sequence
  C25 LC CDR2
LASSLDS

SEQ ID NO: 109 - protein, 10 aa, Artificial Sequence
  C25 LC CDR3
AGGYNGDIYT

SEQ ID NO: 110 - protein, 13 aa, Artificial Sequence
  C7 LC CDR1
QASESVDYNNQLS

SEQ ID NO: 111 - protein, 7 aa, Artificial Sequence
  C7 LC CDR2
YVSTLDS

SEQ ID NO: 112 - protein, 10 aa, Artificial Sequence
  C7 LC CDR3
QGGYPYNIYP

SEQ ID NO: 113 - protein, 13 aa, Artificial Sequence
  C6 LC CDR1
QSSESVDYNNQLS

SEQ ID NO: 114 - protein, 7 aa, Artificial Sequence
  C6 LC CDR2
YVSTLDS

SEQ ID NO: 115 - protein, 10 aa, Artificial Sequence
  C6 LC CDR3
QGGYISNIYP

SEQ ID NO: 116 - protein, 13 aa, Artificial Sequence
  C1 LC CDR1
QSSESVDNNNQLS

SEQ ID NO: 117 - protein, 7 aa, Artificial Sequence
  C1 LC CDR2
YVSTLDS

SEQ ID NO: 118 - protein, 10 aa, Artificial Sequence
  C1 LC CDR3
QGGYISNLYP

SEQ ID NO: 119 - protein, 13 aa, Artificial Sequence
  C16 LC CDR1
QSSESVGMNNQLS

SEQ ID NO: 120 - protein, 7 aa, Artificial Sequence
  C16 LC CDR2
YVSTLDS

SEQ ID NO: 121 - protein, 10 aa, Artificial Sequence
  C16 LC CDR3
QGGYISNLYP

SEQ ID NO: 122 - protein, 13 aa, Artificial Sequence
  C20 LC CDR1
QSSESVDMNNQLS

SEQ ID NO: 123 - protein, 7 aa, Artificial Sequence
  C20 LC CDR2
YVSTLDS

SEQ ID NO: 124 - protein, 10 aa, Artificial Sequence
  C20 LC CDR3
QGGYISNLYP

SEQ ID NO: 125 - protein, 13 aa, Artificial Sequence
  C22 LC CDR1
QSSESVDMNNQLS

SEQ ID NO: 126 - protein, 7 aa, Artificial Sequence
  C22 LC CDR2
YVSTLDS

SEQ ID NO: 127 - protein, 10 aa, Artificial Sequence
  C22 LC CDR3
QGGYISNLYP

SEQ ID NO: 128 - protein, 13 aa, Artificial Sequence
  C10 LC CDR1
QSSESVDYGNQLS

SEQ ID NO: 129 - protein, 7 aa, Artificial Sequence
  C10 LC CDR2
YVSILDA

SEQ ID NO: 130 - protein, 10 aa, Artificial Sequence
  C10 LC CDR3
QGGYISNLYP

SEQ ID NO: 131 - protein, 13 aa, Artificial Sequence
  C12 LC CDR1
QSSESVDYGNQLS

SEQ ID NO: 132 - protein, 7 aa, Artificial Sequence
  C12 LC CDR2
YVSILDA

SEQ ID NO: 133 - protein, 10 aa, Artificial Sequence
  C12 LC CDR3
QGGYISNLYP

SEQ ID NO: 134 - protein, 13 aa, Artificial Sequence
  C13 LC CDR1
QSSESVDNNNQLS

SEQ ID NO: 135 - protein, 7 aa, Artificial Sequence
  C13 LC CDR2
YASTLDS

SEQ ID NO: 136 - protein, 10 aa, Artificial Sequence
  C13 LC CDR3
QGGTATNIYP

SEQ ID NO: 137 - protein, 13 aa, Artificial Sequence
  C14 LC CDR1
QSSESVDYNNQLS

SEQ ID NO: 138 - protein, 7 aa, Artificial Sequence
  C14 LC CDR2
YVSTLDS

SEQ ID NO: 139 - protein, 10 aa, Artificial Sequence
  C14 LC CDR3
QGGYISNLYP

SEQ ID NO: 140 - protein, 13 aa, Artificial Sequence
  C11 LC CDR1
QSSESVDYNNQLS

SEQ ID NO: 141 - protein, 7 aa, Artificial Sequence
  C11 LC CDR2
YVSTLDS

SEQ ID NO: 142 - protein, 10 aa, Artificial Sequence
  C11 LC CDR3
QGGYISNLYP

SEQ ID NO: 143 - protein, 13 aa, Artificial Sequence
  C4 LC CDR1
QASQSIYNNNQLS

SEQ ID NO: 144 - protein, 7 aa, Artificial Sequence
  C4 LC CDR2
YASTLAS

SEQ ID NO: 145 - protein, 13 aa, Artificial Sequence
  C4 LC CDR3
QGQFNCRSADCHA

SEQ ID NO: 146 - protein, 12 aa, Artificial Sequence
  C5 LC CDR1
QSSQSVWSNYLS

SEQ ID NO: 147 - protein, 7 aa, Artificial Sequence
  C5 LC CDR2
GTSKLPS

SEQ ID NO: 148 - protein, 10 aa, Artificial Sequence
  C5 LC CDR3
AGGYSGHIYS

SEQ ID NO: 149 - protein, 11 aa, Artificial Sequence
  C9 LC CDR1
QASQSINSWLS

SEQ ID NO: 150 - protein, 7 aa, Artificial Sequence
  C9 LC CDR2
GASNLAS

SEQ ID NO: 151 - protein, 15 aa, Artificial Sequence
  C9 LC CDR3
LGYYYSSYNSVGFWA

SEQ ID NO: 152 - protein, 13 aa, Artificial Sequence
  C26 LC CDR1
QASQSVYNNNDLA

SEQ ID NO: 153 - protein, 7 aa, Artificial Sequence
  C26 LC CDR2
EASKLAS

SEQ ID NO: 154 - protein, 10 aa, Artificial Sequence
  C26 LC CDR3
AGGWSGNFYV

SEQ ID NO: 155 - protein, 13 aa, Artificial Sequence
  C27 LC CDR1
QASQSVYDGNWLC

SEQ ID NO: 156 - protein, 7 aa, Artificial Sequence
  C27 LC CDR2
KASTLES

SEQ ID NO: 157 - protein, 10 aa, Artificial Sequence
  C27 LC CDR3
QGGFTSNIYP

SEQ ID NO: 158 - protein, 13 aa, Artificial Sequence
  C17 LC CDR1
QSSQSVYNNNWLA

SEQ ID NO: 159 - protein, 7 aa, Artificial Sequence
  C17 LC CDR2
GTSELAS

SEQ ID NO: 160 - protein, 10 aa, Artificial Sequence
  C17 LC CDR3
LGTYSSNIHV

SEQ ID NO: 161 - protein, 18 aa, Artificial Sequence
  Cys-apelin-17
CKFRRQRPRLSHKGPMPF

SEQ ID NO: 162 - protein, 14 aa, Artificial Sequence
  pyr-apelin-13-Cys
  MISC_FEATURE (1)..(1): Glu is a pyroglutamic acid
ERPRLSHKGPMPFC

SEQ ID NO: 163 - protein, 13 aa, Artificial Sequence
  pyr-apelin-13
  MISC_FEATURE (1)..(1): Glu is a pyroglutamic acid
ERPRLSHKGPMPF

SEQ ID NO: 164 - protein, 14 aa, Artificial Sequence
  Cys(Q) apelin-13
CQRPRLSHKGPMPF

SEQ ID NO: 165 - protein, 13 aa, Artificial Sequence
  biotin-apelin-13
QRPRLSHKGPMPF

SEQ ID NO: 166 - protein, 17 aa, Artificial Sequence
  biotin-apelin-17
KFRRQRPRLSHKGPMPF

SEQ ID NO: 167 - protein, 14 aa, Artificial Sequence
  biotin-apelin-(27-14)
GPGAWQGGRRKFRR

SEQ ID NO: 168 - protein, 5 aa, Artificial Sequence
  HC CDR1
  MISC_FEATURE (1)..(1): Xaa is Ser or Thr
  MISC_FEATURE (4)..(4): Xaa is Met or Val
XRNXS

SEQ ID NO: 169 - protein, 14 aa, Artificial Sequence
  HC CDR2
  MISC_FEATURE (8)..(8): Xaa is Tyr or Phe
  MISC_FEATURE (13)..(13): Xaa is Lys or Gln
SIGSSPWXASWAXG

SEQ ID NO: 170 - protein, 9 aa, Artificial Sequence
  HC CDR3
  MISC_FEATURE (7)..(7): Xaa is Ala and Gly
  MISC_FEATURE (9)..(9): Xaa is Val or Ile
GGYRPGXSX

SEQ ID NO: 171 - protein, 13 aa, Artificial Sequence
  LC CDR1
  MISC_FEATURE (13)..(13): Xaa is Ala or Gly
QSSQSVYDNNDLX

SEQ ID NO: 172 - protein, 10 aa, Artificial Sequence
  LC CDR3
  MISC_FEATURE (5)..(5): Xaa is Ser or Asn
AGGYXGDIYT

SEQ ID NO: 173 - protein, 5 aa, Artificial Sequence
  HC CDR1
  MISC_FEATURE (1)..(1): Xaa is Asn or Ser
  MISC_FEATURE (4)..(4): Xaa is Met or Ile
XYAXD

SEQ ID NO: 174 - protein, 16 aa, Artificial Sequence
  HC CDR2
  MISC_FEATURE (6)..(6): Xaa is Arg, Gly, or His
  MISC_FEATURE (7)..(7): Xaa is Arg, Ala, or Tyr
  MISC_FEATURE (9)..(9): Xaa is Tyr or Cys
VIAPNXXTXYPTWARG

SEQ ID NO: 175 - protein, 9 aa, Artificial Sequence
  HC CDR3
  MISC_FEATURE (4)..(4): Xaa is Glu or Asp
  MISC_FEATURE (5)..(5): Xaa is Pro, Ala, Ser, or Thr
  MISC_FEATURE (7)..(7): Xaa is Ala or Ser
YPIXXGXNI

SEQ ID NO: 176 - protein, 13 aa, Artificial Sequence
  LC CDR1
  MISC_FEATURE (7)..(7): Xaa is Asp or Gly
  MISC_FEATURE (8)..(8): Xaa is Tyr, Asn, or Met
QSSESVXXNNQLS

SEQ ID NO: 177 - protein, 16 aa, Artificial Sequence
  HC CDR2
  MISC_FEATURE (6)..(6): Xaa is Gly or Ser
VIAPSXTTYYPTWAKG

SEQ ID NO: 178 - protein, 9 aa, Artificial Sequence
  HC CDR2
  MISC_FEATURE (9)..(9): Xaa is Ile or Val
YPIDPGSNX

SEQ ID NO: 179 - protein, 5 aa, Artificial Sequence
  HC CDR1
  MISC_FEATURE (1)..(1): Xaa is Asn or Ser
  MISC_FEATURE (2)..(2): Xaa is Tyr or His
XXAMD

SEQ ID NO: 180 - protein, 9 aa, Artificial Sequence
  HC CDR3
  MISC_FEATURE (5)..(5): Xaa is Val or Ala
YPIDXGANV

SEQ ID NO: 181 - protein, 12 aa, Artificial Sequence
  Apelin Peptide 1-12
QRPRLSHKGPMP

SEQ ID NO: 182 - protein, 12 aa, Artificial Sequence
  Apelin Peptide 2-13
RPRLSHKGPMPF

SEQ ID NO: 183 - protein, 11 aa, Artificial Sequence
  Apelin Peptide 3-13
PRLSHKGPMPF

SEQ ID NO: 184 - protein, 10 aa, Artificial Sequence
  Apelin Peptide 4-13
RLSHKGPMPF

SEQ ID NO: 185 - protein, 9 aa, Artificial Sequence
  Apelin Peptide 5-13
LSHKGPMPF

SEQ ID NO: 186 - protein, 8 aa, Artificial Sequence
  Apelin Peptide 6-13
SHKGPMPF

SEQ ID NO: 187 - protein, 7 aa, Artificial Sequence
  Apelin Peptide 7-13
HKGPMPF

SEQ ID NO: 188 - protein, 6 aa, Artificial Sequence
  Apelin Peptide 8-13
KGPMPF

SEQ ID NO: 189 - protein, 5 aa, Artificial Sequence
  Apelin Peptide 9-13
GPMPF

SEQ ID NO: 190 - protein, 4 aa, Artificial Sequence
  Apelin Peptide 10-13
PMPF

SEQ ID NO: 191 - protein, 3 aa, Artificial Sequence
  Apelin Peptide 11-13
MPF

SEQ ID NO: 192 - protein, 6 aa, Artificial Sequence
  Peptide 8A
AGPMPF

SEQ ID NO: 193 - protein, 6 aa, Artificial Sequence
  Peptide 9A
KAPMPF

SEQ ID NO: 194 - protein, 6 aa, Artificial Sequence
  Peptide 10A
KGAMPF

SEQ ID NO: 195 - protein, 6 aa, Artificial Sequence
  Peptide 11A
KGPAPF

SEQ ID NO: 196 - protein, 6 aa, Artificial Sequence
  Peptide 12A
KGPMAF

SEQ ID NO: 197 - protein, 6 aa, Artificial Sequence
  Peptide 13A
KGPMPA

SEQ ID NO: 198 - protein, 11 aa, Artificial Sequence
  Apelin Peptide 1-11
QRPRLSHKGPM

SEQ ID NO: 199 - protein, 10 aa, Artificial Sequence
  Apelin Peptide 1-10
QRPRLSHKGP

SEQ ID NO: 200 - protein, 9 aa, Artificial Sequence
  Apelin Peptide 1-9
QRPRLSHKG

SEQ ID NO: 201 - protein, 8 aa, Artificial Sequence
  Apelin Peptide 1-8
QRPRLSHK

SEQ ID NO: 202 - protein, 7 aa, Artificial Sequence
  Apelin Peptide 1-7
QRPRLSH

SEQ ID NO: 203 - protein, 6 aa, Artificial Sequence
  Apelin Peptide 1-6
QRPRLS

SEQ ID NO: 204 - protein, 5 aa, Artificial Sequence
  Apelin Peptide 1-5
QRPRL

SEQ ID NO: 205 - protein, 4 aa, Artificial Sequence
  Apelin Peptide 1-4
QRPR

SEQ ID NO: 206 - protein, 5 aa, Artificial Sequence
  1A
ARPRL

SEQ ID NO: 207 - protein, 5 aa, Artificial Sequence
  2A
QAPRL

SEQ ID NO: 208 - protein, 5 aa, Artificial Sequence
  3A
QRARL

SEQ ID NO: 209 - protein, 5 aa, Artificial Sequence
  4A
QRPAL

SEQ ID NO: 210 - protein, 5 aa, Artificial Sequence
  5A
QRPRA

SEQ ID NO: 211 - protein, 113 aa, Artificial Sequence
  Humanized VH
QSLEESGGGLVQPGGSLRLSCAVSGIDLYSNRMSWVRQAPGKGLEWVSSIGSSPWYASWAQGRFTISRDNSNTLYLQMNSLTAEDTAVYYCAKGGYRPGASVWGQGTLVTVSS

SEQ ID NO: 212 - protein, 113 aa, Artificial Sequence
  Humanized VH
QSLEESGGGLVQPGGSLRLSCAVSGIDLYSNRMSWVRQAPGKGLEWVSSIGSSPWYASWAQGRFTISRDNSNTVYLQMNSLTAEDTATYFCAKGGYRPGASVWGQGTLVTVSS

SEQ ID NO: 213 - protein, 113 aa, Artificial Sequence
  Humanized VH
QSLEESGGGLVQPGGSLRLSCAVSGIDLYSNRMSWVRQAPGKGLEWVGSIGSSPWYASWAQGRFTISRDNSNTVYLQMNSLTAEDTATYFCAKGGYRPGASVWGQGTLVTVSS

SEQ ID NO: 214 - protein, 113 aa, Artificial Sequence
  Humanized VH
QSLEESGGGLVQPGGSLRLSCTVSGIDLYSNRMSWVRQAPGKGLEWVGSIGSSPWYASWAQGRFTISRDNSNTVYLKMNSPTAEDTATYFCAKGGYRPGASVWGQGTLVTVSS

SEQ ID NO: 215 - protein, 110 aa, Artificial Sequence
  Humanized VL
DIQLTQSPSSLSASVGDRVTITCQSSQSIYDNNDLAWYQQKPGKTPKRLIYLASSLDSGVPSRFSGSGSGTDFTLTISSLQPEDVATYYCAGGYSGDIYTFGGGTKVEIK

SEQ ID NO: 216 - protein, 110 aa, Artificial Sequence
  Humanized VL
AQVLTQSPSSLSASVGDRVTIACQSSQSVYDNNDLAWYQQKAGQTPKRLIYLASSLDSGVPSRFSGSGSGTEFTLTISSLQCEDVATYYCAGGYSGDIYTFGGGTEVVVE

SEQ ID NO: 217 - protein, 113 aa, Artificial Sequence
  B24 Heavy Chain Variable Region
QSLEESGGGLVQPGGSLRLSCTVSGIDLYTNRVSWVRQAPGKGLEWVGSIGSSPWYASWAQGRFTISRDNSNTVYLKMNSPTAEDTATYFCAKGGYRPGGSIWGQGTLVTVSS

SEQ ID NO: 218 - protein, 113 aa, Artificial Sequence
  B25 Heavy Chain Variable Region
QSLEESGGGLVQPGGSLRLSCTVSGIDLYTNRMSWVRQAPGKGLEWVGSIGSSPWFASWALGRFTISRDNSNTVYLKMNSPTAEDTATYFCAKGGYRPGASVWGQGTLVTVSS

SEQ ID NO: 219 - protein, 110 aa, Artificial Sequence
  B24 Light Chain Variable Region
DIQLTQSPSSLSASVGDRVTITCQSSQSIYDNNDLGWYQQKPGKTPKRLIYLASSLDSGVPSRFSGSGSGTDFTLTISSLQPEDVATYYCAGGYSGDIYTFGGGTKVEIK

SEQ ID NO: 220 - protein, 110 aa, Artificial Sequence
  B25 Light Chain Variable Region
DIQLTQSPSSLSASVGDRVTITCQSSQSIYDNNDLAWYQQKPGKTPKRLIYLASSLDSGVPSRFSGSGSGTDFTLTISSLQPEDVATYYCAGGYNGDIYTFGGGTKVEIK

SEQ ID NO: 221 - protein, 77 aa, Homo sapiens
MNLRLCVQALLLLWLSLTAVCGGSLMPLPDGNGLEDGNVRHLVQPRGSRNGPGPWQGGRRKFRRQRPRLSHKGPMPF